European Patent Application EP 4 151 228 A2, published March 22, 2023. Title: LYSIN POLYPEPTIDES ACTIVE AGAINST GRAM-NEGATIVE BACTERIA. Applicant: CONTRAFECT CORPORATION. Application US 17/811,325, filed July 8, 2022. The sequence listing filed with the application follows.

SEQUENCE LISTING (21 sequences)

SEQ ID NO: 1 - protein, 126 aa, Micavibrio aeruginosavorus
MTYTLSKRSLDNLKGVHPDLVAVVHRAIQLTPVDFAVIEGLRSVSRQKELVAAGASKTMNSRHLTGHAVDLAAYVNGIRWDWPLYDAIAVAVKAAAKELGVAIVWGGDWTTFKDGPHFELDRSKYR

SEQ ID NO: 2 - protein, 147 aa, unidentified
  REGION 1..147: note = hypothetical protein GOS_817346 [marine metagenome] (GenBank:EDG23390.1)
MKISLEGLSLIKKFEGCKLEAYKCSAGVWTIGYGHTAGVKEGDVCTQEEAEKLLRGDIFKFEEYVQDSVKVDLDQSQFDALVAWTFNLGPGNLRSSTMLKKLNNGEYESVPFEMRRWNKAGGKTLDGLIRRRQAESLLFESKEWHQV

SEQ ID NO: 3 - protein, 144 aa, Pseudomonas phage PAJU2
MRTSQRGIDLIKSFEGLRLSAYQDSVGVWTIGYGTTRGVTRYMTITVEQAERMLSNDIQRFEPELDRLAKVPLNQNQWDALMSFVYNLGAANLASSTLLKLLNKGDYQGAADQFPRWVNAGGKRLDGLVKRRAAERALFLEPLS

SEQ ID NO: 4 - protein, 181 aa, Pseudomonas phage Lu11
MNNELPWVAEARKYIGLREDTSKTSHNPKLLAMLDRMGEFSNESRAWWHDDETPWCGLFVGYCLGVAGRYVVREWYRARAWEAPQLTKLDRPAYGALVTFTRSGGGHVGFIVGKDARGNLMVLGGNQSNAVSIAPFAVSRVTGYFWPSFWRNKTAVKSVPFEERYSLPLLKSNGELSTNEA

SEQ ID NO: 5 - protein, 439 aa, Pseudomonas sp.
MKRTTLNLELESNTDRLLQEKDDLLPQSVTNSSDEGTPFAQVEGASDDNTAEQDSDKPGASVADADTKPVDPEWKTITVASGDTLSTVFTKAGLSTSAMHDMLTSSKDAKRFTHLKVGQEVKLKLDPKGELQALRVKQSELETIGLDKTDKGYSFKREKAQIDLHTAYAHGRITSSLFVAGRNAGLPYNLVTSLSNIFGYDIDFALDLREGDEFDVIYEQHKVNGKQVATGNILAARFVNRGKTYTAVRYTNKQGNTSYYRADGSSMRKAFIRTPVDFARISSRFSLGRRHPILNKIRAHKGVDYAAPIGTPIKATGDGKILEAGRKGGYGNAVVIQHGQRYRTIYGHMSRFAKGIRAGTSVKQGQIIGYVGMTGLATGPHLHYEFQINGRHVDPLSAKLPMADPLGGADRKRFMAQTQPMIARMDQEKKTLLALNKQR

SEQ ID NO: 6 - protein, 39 aa, synthetic construct
  REGION 1..39: note = artificially-created modified fragment of GN4 (SEQ ID NO: 3)
NKGDYQGAADQFPRWVNAGGKRLDGLVKRRASQSRESQC

SEQ ID NO: 7 - protein, 42 aa, Pseudomonas phage PAJU2
NKGDYQGAADQFPRWVNAGGKRLDGLVKRRAAERALFLEPLS

SEQ ID NO: 8 - protein, 31 aa, Pseudomonas phage PAJU2
NKGDYQGAADQFPRWVNAGGKRLDGLVKRRA

SEQ ID NO: 9 - protein, 31 aa, synthetic construct
  REGION 1..31: note = artificially-created modified fragment of GN4 (SEQ ID NO: 3)
NKGDYQGAADQFPRWVNAGGKRLDGLVKRRK

SEQ ID NO: 10 - protein, 43 aa, synthetic construct
  REGION 1..43: note = artificially-created modified fragment of GN4 (SEQ ID NO: 3)
NKGDYQGAADQFPRWVNAGGKRLDGLVKRRAAERALFLEPLSC

SEQ ID NO: 11 - DNA, 381 bp, Micavibrio aeruginosavorus
  source 1..381: mol_type = genomic DNA
atgacatacaccctgagcaaaagaagcctggataacctaaaaggcgttcatcccgatctggttgccgttgtccatcgcgccatccagcttacaccggttgatttcgcggtgatcgaaggcctgcgctccgtatcccgccaaaaggaactggtggccgccggcgccagcaagaccatgaacagccgacacctgacaggccatgcggttgatctagccgcttacgtcaatggcatccgctgggactggcccctgtatgacgccatcgccgtggctgtgaaagccgcagcaaaggaattgggtgtggccatcgtgtggggcggtgactggaccacgtttaaggatggcccgcactttgaactggatcggagcaaatacagatga

SEQ ID NO: 12 - DNA, 444 bp, unidentified
  misc_feature 1..444: note = Marine metagenome; polynucleotide sequence for the polypeptide ofSEQ ID NO: 2
  source 1..444: mol_type = genomic DNA
atgaaaattagtttagagggattatctctcatcaaaaaatttgagggttgtaaactagaagcatacaaatgttctgcaggagtgtggactataggttatggtcatactgcaggtgtaaaagaaggtgatgtttgcacacaagaggaagctgaaaaattattaagaggagatatctttaaatttgaagagtatgtgcaagatagtgtaaaggttgatttagaccaaagtcaatttgacgcattagttgcatggacatttaatttaggcccaggtaatttaagaagttcaaccatgttgaaaaaattaaataatggagagtatgaatctgttcctttcgaaatgagaaggtggaataaagcaggtggtaaaaccttagatggtttaatcagaagacgccaagcagaatcattattatttgaaagtaaagagtggcatcaagtataa

SEQ ID NO: 13 - DNA, 435 bp, Pseudomonas phage PAJU2
  source 1..435: mol_type = genomic DNA
atgcgtacatcccaacgaggcatcgacctcatcaaatccttcgagggcctgcgcctgtccgcttaccaggactcggtgggtgtctggaccataggttacggcaccactcggggcgtcacccgctacatgacgatcaccgtcgagcaggccgagcggatgctgtcgaacgacattcagcgcttcgagccagagctagacaggctggcgaaggtgccactgaaccagaaccagtgggatgccctgatgagcttcgtgtacaacctgggcgcggccaatctggcgtcgtccacgctgctcaagctgctgaacaagggtgactaccagggagcagcggaccagttcccgcgctgggtgaatgcgggcggtaagcgcttggatggtctggttaagcgtcgagcagccgagcgtgcgctgttcctggagccactatcgtga

SEQ ID NO: 14 - DNA, 546 bp, Pseudomonas phage Lu11
  source 1..546: mol_type = genomic DNA
atgaataacgaacttccttgggtagccgaagcccgaaagtatatcggccttcgcgaagacacttcgaagacttcgcataacccgaaacttcttgccatgcttgaccgcatgggcgaattttccaacgaatcccgcgcttggtggcacgacgacgaaacgccttggtgcggactgttcgtcggctattgcttgggcgttgccgggcgctacgtcgtccgcgaatggtacagggcgcgggcatgggaagccccgcagcttacgaagcttgaccggcccgcatacggcgcgcttgtgaccttcacgcgaagcggcggcggccacgtcggttttattgtgggcaaggatgcgcgcggaaatcttatggttcttggcggtaatcagtcgaacgccgtaagtatcgcaccgttcgcagtatcccgcgtaaccggctatttctggccgtcgttctggcgaaacaagaccgcagttaaaagcgttccgtttgaagaacgttattcgctgccgctgttgaagtcgaacggcgaactttcgacgaatgaagcgtaa

SEQ ID NO: 15 - DNA, 546 bp, Pseudomonas sp.; identical to SEQ ID NO: 14
  source 1..546: mol_type = genomic DNA

SEQ ID NO: 16 - protein, 8 aa, Hepatitis B virus
SQSRESQC

SEQ ID NO: 17 - DNA, 1320 bp, Pseudomonas sp.
  source 1..1320: mol_type = genomic DNA
atgaagaggaccacgctcaatctggagcttgaaagcaacaccgatcgcctccttcaggagaaagacgacctcctgccgcaatcggtcaccaattccagcgacgaaggcacgcctttcgctcaggtagaaggcgcctccgacgacaacaccgccgagcaagactcggacaagccgggcgcatctgtagccgatgccgacaccaagcccgtcgatcccgagtggaagaccatcaccgtcgccagtggcgatacgctgtcgaccgtattcaccaaggcaggcctttccacctcggccatgcacgacatgctgaccagcagcaaggatgccaagcgcttcacccatctgaaggtcggccaggaggtcaagctcaagctcgaccccaaaggagagctgcaggcactgcgagtcaagcagagcgaactcgagaccatcggcctggacaagaccgacaagggctactccttcaaacgcgagaaggcccagatcgacctgcataccgcctatgcccatggccgcatcaccagctcgctgttcgttgccggtcgtaacgccggcctgccctataacctggtcacgtcgctgtcgaacatcttcggctacgacatcgacttcgccctcgatctgcgtgaaggcgacgagttcgacgtgatctacgaacaacacaaggtcaacggcaagcaagtggcgaccggcaatatcctcgccgcccgcttcgtcaaccgtggcaagacctacaccgccgtgcgctataccaacaagcagggcaataccagctactaccgcgccgacggctccagcatgcgcaaggcattcatccgtacgccggtggatttcgcccgtatcagctcgcgcttctccctgggccgccgccacccgatcctgaacaagatccgcgcacacaagggcgtcgactacgcagcccccatcggcacaccgatcaaggccaccggagacggcaagatcctcgaagccggacgcaaggggggctacggcaacgccgtggtgatccagcacggccagcgctatcggaccatctacggacacatgagccgcttcgccaagggtatccgcgccggtaccagcgtgaagcagggccagatcatcggttacgtaggcatgacgggcctggccaccggcccgcacctgcactacgagttccagatcaatggccgtcacgtcgatccgctgagcgccaagctgcccatggcggacccgctcggtggcgcagatcgcaagcgcttcatggcgcagacccagccgatgatcgcgcgcatggatcaggagaagaaaaccctcctggccctgaacaagcagcgctga

SEQ ID NO: 18 - protein, 127 aa, Streptomyces sp. 212
MSFGLSQRSRERLKGVHPDLVAVVEAAIRLTPVDFMITEGLRTPARQAELVRAGASRTLNSRHLTGHAVDVAAWIDGEVRWDWPLYPRIAEAFKAAAKDRDVALIWGGDWPRLRDGPHFELDRRGYP

SEQ ID NO: 19 - protein, 125 aa, Escherichia coli
MPGKFRFSRRSEKNLEGVKPQLVAVVRRALELTEVDFGITEGLRSKYRQKQLVAAGKSQTMNSRHLTGDAVDVVAYIGSQVSWDWPLYEKIAQAFKQAAAELGTAIEWGGDWKTLKDGPHFQLKR

SEQ ID NO: 20 - protein, 125 aa, Enterobacteria phage phiP27
MSGKFRFSRRSEKNLEGVKPQLVAVVRRALELTEVDFGITEGLRTKERQKQLVAEGKSQTMNSRHLTGDAVDVVAYIGSQVSWDWPLYEKIAQAFKQAAAELGTAIEWGGDWKTLKDGPHFQLKW

SEQ ID NO: 21 - protein, 138 aa, Yersinia phage PY100
MEVQPTIEEVSMGFKLGSRSLQRLQGVHPDLVKVVKRAIEISPVDFTVTEGLRTLERQKELFAKGASKTMRSRHLTGHAVDISPLVDGKVSWDWKYYYPMADAMKQAAKELNIPVEWGGDWKTFKDGPHFQLPYGVYK